European Patent Application EP 4 509 524 A1, published February 19, 2025. Title: 增强细胞功能的CD16抗剪切突变体. Applicant: 星奕昂（上海）生物科技有限公司. The sequence listing filed with the application follows.

SEQUENCE LISTING (6 sequences)

SEQ ID NO: 1 - protein, 254 aa, synthetic construct
  source 1..254: note = CD16-WT
MWQLLLPTALLLLVSAGMRTEDLPKAVVFLEPQWYRVLEKDSVTLKCQGAYSPEDNSTQWFHNESLISSQASSYFIDAATVDDSGEYRCQTNLSTLSDPVQLEVHIGWLLLQAPRWVFKEEDPIHLRCHSWKNTALHKVTYLQNGKGRKYFHHNSDFYIPKATLKDSGSYFCRGLFGSKNVSSETVNITITQGLAVSTISSFFPPGYQVSFCLVMVLLFAVDTGLYFSVKTNIRSSTRDWKDHKFKWRKDPQDK

SEQ ID NO: 2 - protein, 254 aa, synthetic construct
  source 1..254: note = CD16-F176V-S197P(PC)
MWQLLLPTALLLLVSAGMRTEDLPKAVVFLEPQWYRVLEKDSVTLKCQGAYSPEDNSTQWFHNESLISSQASSYFIDAATVDDSGEYRCQTNLSTLSDPVQLEVHIGWLLLQAPRWVFKEEDPIHLRCHSWKNTALHKVTYLQNGKGRKYFHHNSDFYIPKATLKDSGSYFCRGLVGSKNVSSETVNITITQGLAVPTISSFFPPGYQVSFCLVMVLLFAVDTGLYFSVKTNIRSSTRDWKDHKFKWRKDPQDK

SEQ ID NO: 3 - protein, 255 aa, synthetic construct
  source 1..255: note = CD16-F176V -V196_S197insP Mut1
MWQLLLPTALLLLVSAGMRTEDLPKAVVFLEPQWYRVLEKDSVTLKCQGAYSPEDNSTQWFHNESLISSQASSYFIDAATVDDSGEYRCQTNLSTLSDPVQLEVHIGWLLLQAPRWVFKEEDPIHLRCHSWKNTALHKVTYLQNGKGRKYFHHNSDFYIPKATLKDSGSYFCRGLVGSKNVSSETVNITITQGLAVPSTISSFFPPGYQVSFCLVMVLLFAVDTGLYFSVKTNIRSSTRDWKDHKFKWRKDPQDK

SEQ ID NO: 4 - protein, 255 aa, synthetic construct
  source 1..255: note = CD16-F176V -S197_T198insP Mut2
MWQLLLPTALLLLVSAGMRTEDLPKAVVFLEPQWYRVLEKDSVTLKCQGAYSPEDNSTQWFHNESLISSQASSYFIDAATVDDSGEYRCQTNLSTLSDPVQLEVHIGWLLLQAPRWVFKEEDPIHLRCHSWKNTALHKVTYLQNGKGRKYFHHNSDFYIPKATLKDSGSYFCRGLVGSKNVSSETVNITITQGLAVSPTISSFFPPGYQVSFCLVMVLLFAVDTGLYFSVKTNIRSSTRDWKDHKFKWRKDPQDK

SEQ ID NO: 5 - protein, 256 aa, synthetic construct
  source 1..256: note = CD16-F176V -V196_S197insP-V197_T198insP Mut3
MWQLLLPTALLLLVSAGMRTEDLPKAVVFLEPQWYRVLEKDSVTLKCQGAYSPEDNSTQWFHNESLISSQASSYFIDAATVDDSGEYRCQTNLSTLSDPVQLEVHIGWLLLQAPRWVFKEEDPIHLRCHSWKNTALHKVTYLQNGKGRKYFHHNSDFYIPKATLKDSGSYFCRGLVGSKNVSSETVNITITQGLAVPSPTISSFFPPGYQVSFCLVMVLLFAVDTGLYFSVKTNIRSSTRDWKDHKFKWRKDPQDK

SEQ ID NO: 6 - protein, 254 aa, synthetic construct
  source 1..254: note = CD16-F176V
MWQLLLPTALLLLVSAGMRTEDLPKAVVFLEPQWYRVLEKDSVTLKCQGAYSPEDNSTQWFHNESLISSQASSYFIDAATVDDSGEYRCQTNLSTLSDPVQLEVHIGWLLLQAPRWVFKEEDPIHLRCHSWKNTALHKVTYLQNGKGRKYFHHNSDFYIPKATLKDSGSYFCRGLVGSKNVSSETVNITITQGLAVSTISSFFPPGYQVSFCLVMVLLFAVDTGLYFSVKTNIRSSTRDWKDHKFKWRKDPQDK